European Patent Specification EP 4 065 978 B1, published December 13, 2023. Title: Novel Linker Compounds. Applicant: Cambridge Enterprise Limited. The sequence listing filed with the application follows.

SEQUENCE LISTING (7 sequences)

SEQ ID NO: 1 - DNA, 39 bp, Artificial Sequence
  ON sequence 1
tttttgatccgattggaaccgtcccaagcgttgcgctag

SEQ ID NO: 2 - DNA, 39 bp, Artificial Sequence
  ON sequence 2
tttttgctatcgttcgttcgaggccagagcattcgctag

SEQ ID NO: 3 - DNA, 60 bp, Artificial Sequence
  Histone H3 (D1h2) XP(R) associated ON
  misc_feature (1)..(1): /5AzideN/
agaggcggccaatacaagccgggatgtattgaaggaggatagaggcggccaatacaagcc

SEQ ID NO: 4 - DNA, 60 bp, Artificial Sequence
  Cleaved Caspase-3 associated ON
  misc_feature (1)..(1): /5AzideN/
agaggcggccaatacaagccagagtgagtagtagtggagtagaggcggccaatacaagcc

SEQ ID NO: 5 - DNA, 60 bp, Artificial Sequence
  Anti-CD44 associated ON
  misc_feature (1)..(1): /5AzideN/
agaggcggccaatacaagcctgtgatggaagttagagggtagaggcggccaatacaagcc

SEQ ID NO: 6 - DNA, 60 bp, Artificial Sequence
  Anti-DNA/RNA G-quadruplex (BG4) associated ON
  misc_feature (1)..(1): /5AzideN/
agaggcggccaatacaagccaggttaggttgagaataggaagaggcggccaatacaagcc

SEQ ID NO: 7 - DNA, 60 bp, Artificial Sequence
  Anti-CD31 associated ON
  misc_feature (1)..(1): /5AzideN/
agaggcggccaatacaagccgatgatgtagtagtaagggtagaggcggccaatacaagcc